European Patent Specification EP 3 825 689 B1, published July 22, 2026. Title: A cell-based method for determining an activity of botulinum toxin. Applicant: Hugel Inc. The sequence listing filed with the application follows.

SEQUENCE LISTING (90 sequences)

SEQ ID NO: 1 - protein, 13 aa, clostridium botulinum
MAEDADMRNELEE

SEQ ID NO: 2 - protein, 13 aa, clostridium botulinum
MAEDADMRNELEE

SEQ ID NO: 3 - protein, 20 aa, clostridium botulinum
DQLADESLESTRRMLQLVEE

SEQ ID NO: 4 - protein, 20 aa, clostridium botulinum
DEQGEQLERIEEGMDQINKD

SEQ ID NO: 5 - protein, 15 aa, clostridium botulinum
DEREQMAISGGFIRR

SEQ ID NO: 6 - protein, 15 aa, clostridium botulinum
EIDTQNRQIDRIMEK

SEQ ID NO: 7 - protein, 15 aa, clostridium botulinum
RIMEKADSNKTRIDE

SEQ ID NO: 8 - protein, 18 aa, clostridium botulinum
RIMEKADSNKTRIDEANQ

SEQ ID NO: 9 - protein, 12 aa, clostridium botulinum
DSNKTRIDEANQ

SEQ ID NO: 10 - protein, 13 aa, clostridium botulinum
KTRIDEANQPATK

SEQ ID NO: 11 - protein, 9 aa, Artificial Sequence
  antibody CDR of clostridium botulinum
GYSITSGYY

SEQ ID NO: 12 - protein, 8 aa, Artificial Sequence
  antibody CDR of clostridium botulinum
GYTFTDYN

SEQ ID NO: 13 - protein, 8 aa, Artificial Sequence
  antibody CDR of clostridium botulinum
GYTFTNYG

SEQ ID NO: 14 - protein, 7 aa, Artificial Sequence
  antibody CDR of clostridium botulinum
IRYDGSN

SEQ ID NO: 15 - protein, 8 aa, Artificial Sequence
  antibody CDR of clostridium botulinum
IYPYNGDT

SEQ ID NO: 16 - protein, 8 aa, Artificial Sequence
  antibody CDR of clostridium botulinum
INTYTGEP

SEQ ID NO: 17 - protein, 12 aa, Artificial Sequence
  antibody CDR of clostridium botulinum
ARDRDSSYYFDY

SEQ ID NO: 18 - protein, 6 aa, Artificial Sequence
  antibody CDR of clostridium botulinum
VRSGDY

SEQ ID NO: 19 - protein, 7 aa, Artificial Sequence
  antibody CDR of clostridium botulinum
ARGYYDY

SEQ ID NO: 20 - protein, 6 aa, Artificial Sequence
  antibody CDR of clostridium botulinum
DHINNW

SEQ ID NO: 21 - protein, 11 aa, Artificial Sequence
  antibody CDR of clostridium botulinum
QSLLDSNGKTY

SEQ ID NO: 22 - protein, 11 aa, Artificial Sequence
  antibody CDR of clostridium botulinum
QSLLDSDGKTY

SEQ ID NO: 23 - protein, 3 aa, Artificial Sequence
  antibody CDR of clostridium botulinum
DTT

SEQ ID NO: 24 - protein, 3 aa, Artificial Sequence
  antibody CDR of clostridium botulinum
LVS

SEQ ID NO: 25 - protein, 9 aa, Artificial Sequence
  antibody CDR of clostridium botulinum
QQYWSAPPT

SEQ ID NO: 26 - protein, 9 aa, Artificial Sequence
  antibody CDR of clostridium botulinum
WQGTLFPYT

SEQ ID NO: 27 - protein, 9 aa, Artificial Sequence
  antibody CDR of clostridium botulinum
WQGTHFPRT

SEQ ID NO: 28 - protein, 9 aa, Artificial Sequence
  antibody CDR of clostridium botulinum
GYSITSDYA

SEQ ID NO: 29 - protein, 8 aa, Artificial Sequence
  antibody CDR of clostridium botulinum
GFTFNTNA

SEQ ID NO: 30 - protein, 8 aa, Artificial Sequence
  antibody CDR of clostridium botulinum
GYTFTNYT

SEQ ID NO: 31 - protein, 8 aa, Artificial Sequence
  antibody CDR of clostridium botulinum
GYTFNTYA

SEQ ID NO: 32 - protein, 8 aa, Artificial Sequence
  antibody CDR of clostridium botulinum
GFTFSNYG

SEQ ID NO: 33 - protein, 8 aa, Artificial Sequence
  antibody CDR of clostridium botulinum
GFTFNTYA

SEQ ID NO: 34 - protein, 7 aa, Artificial Sequence
  antibody CDR of clostridium botulinum
ISYSVGT

SEQ ID NO: 35 - protein, 10 aa, Artificial Sequence
  antibody CDR of clostridium botulinum
IRSKSNNYAT

SEQ ID NO: 36 - protein, 10 aa, Artificial Sequence
  antibody CDR of clostridium botulinum
IRSKSDNYAT

SEQ ID NO: 37 - protein, 8 aa, Artificial Sequence
  antibody CDR of clostridium botulinum
INPSSDYT

SEQ ID NO: 38 - protein, 10 aa, Artificial Sequence
  antibody CDR of clostridium botulinum
IRSKSNNYTT

SEQ ID NO: 39 - protein, 8 aa, Artificial Sequence
  antibody CDR of clostridium botulinum
INSNGGTT

SEQ ID NO: 40 - protein, 10 aa, Artificial Sequence
  antibody CDR of clostridium botulinum
ARKGEYGFAY

SEQ ID NO: 41 - protein, 11 aa, Artificial Sequence
  antibody CDR of clostridium botulinum
VYGRSYGGLSY

SEQ ID NO: 42 - protein, 11 aa, Artificial Sequence
  antibody CDR of clostridium botulinum
VYGRSYGGLGY

SEQ ID NO: 43 - protein, 13 aa, Artificial Sequence
  antibody CDR of clostridium botulinum
VRQVTTAVGGFAY

SEQ ID NO: 44 - protein, 16 aa, Artificial Sequence
  antibody CDR of clostridium botulinum
ARRIFYNGRTYAAMDY

SEQ ID NO: 45 - protein, 17 aa, Artificial Sequence
  antibody CDR of clostridium botulinum
VGQILYYYVGSPAWFAY

SEQ ID NO: 46 - protein, 9 aa, Artificial Sequence
  antibody CDR of clostridium botulinum
ARDRDAMDY

SEQ ID NO: 47 - protein, 10 aa, Artificial Sequence
  antibody CDR of clostridium botulinum
KSVSTSGYSY

SEQ ID NO: 48 - protein, 10 aa, Artificial Sequence
  antibody CDR of clostridium botulinum
KSVSSSGYSY

SEQ ID NO: 49 - protein, 11 aa, Artificial Sequence
  antibody CDR of clostridium botulinum
QSIVNSHGNTY

SEQ ID NO: 50 - protein, 3 aa, Artificial Sequence
  antibody CDR of clostridium botulinum
LAS

SEQ ID NO: 51 - protein, 3 aa, Artificial Sequence
  antibody CDR of clostridium botulinum
KVS

SEQ ID NO: 52 - protein, 9 aa, Artificial Sequence
  antibody CDR of clostridium botulinum
QHSRELPLT

SEQ ID NO: 53 - protein, 9 aa, Artificial Sequence
  antibody CDR of clostridium botulinum
QHSRELPWT

SEQ ID NO: 54 - protein, 9 aa, Artificial Sequence
  antibody CDR of clostridium botulinum
FQGSHVPWT

SEQ ID NO: 55 - protein, 8 aa, Artificial Sequence
  antibody CDR of clostridium botulinum
GFTFSNYG

SEQ ID NO: 56 - protein, 8 aa, Artificial Sequence
  antibody CDR of clostridium botulinum
GINIKDYY

SEQ ID NO: 57 - protein, 8 aa, Artificial Sequence
  antibody CDR of clostridium botulinum
ISSGGSYT

SEQ ID NO: 58 - protein, 8 aa, Artificial Sequence
  antibody CDR of clostridium botulinum
IDPGNGDA

SEQ ID NO: 59 - protein, 13 aa, Artificial Sequence
  antibody CDR of clostridium botulinum
ARHEGGGNPYFDY

SEQ ID NO: 60 - protein, 5 aa, Artificial Sequence
  antibody CDR of clostridium botulinum
NEIAY

SEQ ID NO: 61 - protein, 11 aa, Artificial Sequence
  antibody CDR of clostridium botulinum
QSLVHSNGNTY

SEQ ID NO: 62 - protein, 11 aa, Artificial Sequence
  antibody CDR of clostridium botulinum
QSLLDSDGKTY

SEQ ID NO: 63 - protein, 3 aa, Artificial Sequence
  antibody CDR of clostridium botulinum
KVS

SEQ ID NO: 64 - protein, 3 aa, Artificial Sequence
  antibody CDR of clostridium botulinum
LVS

SEQ ID NO: 65 - protein, 9 aa, Artificial Sequence
  antibody CDR of clostridium botulinum
SQNTLVPWT

SEQ ID NO: 66 - protein, 9 aa, Artificial Sequence
  antibody CDR of clostridium botulinum
WQGTHFPFT

SEQ ID NO: 67 - protein, 120 aa, Artificial Sequence
  antibody of clostridium botulinum
EVKLVESGGGLVKPGGSLKLSCAASGFTFSNYGMSWVRQTPEKRLEWVATISSGGSYTYYPDSVKGRFTISRDNAKNTLYLQMSSLRSEDTAMYYCARHEGGGNPYFDYWGQGTTLTVSS

SEQ ID NO: 68 - protein, 112 aa, Artificial Sequence
  antibody of clostridium botulinum
DVLMTQTPLSLPVSLGDQASISCRSSQSLVHSNGNTYLHWYLQKPGQSPKLLIYKVSNRFSGVPDRFSGSGSGTDFTLKISRVEAEDLGVYFCSQNTLVPWTFGGGTKLEIK

SEQ ID NO: 69 - protein, 112 aa, Artificial Sequence
  antibody of clostridium botulinum
EVQLQQSGAELVRPGASVKLSCTASGINIKDYYMHWMKQRPEQDLEWIGWIDPGNGDAEYAPKFQGKATMTADTSSNTAYLQLSSLTSEDTAVYYCNEIAYWGQGTLVTVSA

SEQ ID NO: 70 - protein, 112 aa, Artificial Sequence
  antibody of clostridium botulinum
DIVMTQSPLTLSVTIGQPASISCKSSQSLLDSDGKTYLNWLLQRPGQSPKRLIYLVSKLDSGVPDRFTGSGSGTDFTLKISRVEAEDLGVYYCWQGTHFPFTFGSGTKLEIK

SEQ ID NO: 71 - protein, 117 aa, Artificial Sequence
  antibody of clostridium botulinum
DVKLQESGPGLVKPSQSLSLTCTVTGYSITSDYAWNWIRQFPGNKLEWMGYISYSVGTRYNPSLKSRISITRDTSKNQFFLLLKSVTNEDTATYFCARKGEYGFAYWGQGTLVTVSA

SEQ ID NO: 72 - protein, 111 aa, Artificial Sequence
  antibody of clostridium botulinum
DIVMTQSPASLAVSLGQRATISCRASKSVSTSGYSYMHWYQQKPGQPPKLLIYLASNLESGVPARFSGSGSGTDFTLNIHPVEEEDAATYYCQHSRELPLTFGAGTKLELK

SEQ ID NO: 73 - protein, 120 aa, Artificial Sequence
  antibody of clostridium botulinum
QVQLVETGGGLVQPKGSLKLSCAASGFTFNTNAMNWVRQAPGKGLEWVARIRSKSNNYATYYADSVKDRFTISRDDSQSLLYLQMNNLKTEDTAMYYCVYGRSYGGLSYWGQGTLVTVSA

SEQ ID NO: 74 - protein, 111 aa, Artificial Sequence
  antibody of clostridium botulinum
DIVMTQSPASLAVSLGQRATISCRASKSVSSSGYSYMHWYQQKPGQPPKLLIYLASNLESGVPARFSGSGSGTDFTLNIHPVEEEDAATYYCQHSRELPLTFGAGTKLELK

SEQ ID NO: 75 - protein, 120 aa, Artificial Sequence
  antibody of clostridium botulinum
EVKLVESGGGLVQPKGSLKLSCAASGFTFNTNAMNWVRQAPGKGLEWVARIRSKSDNYATYYADSVKDRFTISRDDSPSMLYLQMNNLKTEDTAMYYCVYGRSYGGLGYWGQGTLVTVSA

SEQ ID NO: 76 - protein, 111 aa, Artificial Sequence
  antibody of clostridium botulinum
DIVLTQSPASLAVSLGQRATISCRASKSVSTSGYSYVHWYQQKPGQPPKLLIYLASNLESGVPARFSGSGSGTDFTLNIHPVEEEDAATYYCQHSRELPLTFGAGTKLELK

SEQ ID NO: 77 - protein, 122 aa, Artificial Sequence
  antibody of clostridium botulinum
EVKLVESGGGLVQPKGSLKLSCAASGFTFNTYAMNWVRQAPGKGLEWVARIRSKSNNYATYYADSVKDRFTISRDDSQSMLYLQMNNLKTEDTAMYYCVRQVTTAVGGFAYWGQGTLVTVSE

SEQ ID NO: 78 - protein, 111 aa, Artificial Sequence
  antibody of clostridium botulinum
DIVMTQSPASLAVSLGQRTTISCRASKSVSSSGYSYMHWYQQKPGQPPKLLIYLASNLESGVPARFSGSGSGTDFTLNIHPVEEEDAATYYCQHSRELPLTFGAGTKLELR

SEQ ID NO: 79 - protein, 123 aa, Artificial Sequence
  antibody of clostridium botulinum
EVQLQQSGAELARPGASVQMSCKAFGYTFTNYTMHWVRQRPGQGLEWIGFINPSSDYTNYNQKFKDKATLSADKSSSTAYMQLSSLTSEDSAVYYCARRIFYNGRTYAAMDYWGQGTSVTVSS

SEQ ID NO: 80 - protein, 111 aa, Artificial Sequence; identical to SEQ ID NO: 74
  antibody of clostridium botulinum

SEQ ID NO: 81 - protein, 126 aa, Artificial Sequence
  antibody of clostridium botulinum
EVKLVESGGGLVQPKGSLKLSCAASGYTFNTYAMNWVRQAPGKGLEWVARIRSKSNNYTTYYADSVKDRFTISRDDSQSMLYLQINNLKTEDTAMYYCVGQILYYYVGSPAWFAYWGQGTLVTVSA

SEQ ID NO: 82 - protein, 111 aa, Artificial Sequence
  antibody of clostridium botulinum
DIVMTQSPASLAVSLGQRATISCRASKSVSTSGYSYMHWYQQKPGQPPKLLIFLASNLESGVPARFSGSGSGTDFTLNIHPVEEEDAATYYCQHSRELPWTFGGGTKLEIK

SEQ ID NO: 83 - protein, 119 aa, Artificial Sequence
  antibody of clostridium botulinum
DVKLQESGPGLVKPSQSLSLTCSVTGYSITSGYYWNWIRQFPGNKLEWMGYIRYDGSNNYNPSLKNRISITRDTSKNQFFLKLNSVTTEDTASYYCARDRDSSYYFDYWGQGTALTVSS

SEQ ID NO: 84 - protein, 107 aa, Artificial Sequence
  antibody of clostridium botulinum
DIVMTQSSSYLSVSLGGRVTITCKASDHINNWLAWYQQKPGNAPRLLISDTTSLETGVPSRFSGSGSGKDYTLSITSLQTEDVATYYCQQYWSAPPTFGGGTKLEIK

SEQ ID NO: 85 - protein, 116 aa, Artificial Sequence
  antibody of clostridium botulinum
EVQLEESGGGLVQPGGSLKLSCAASGFTFSNYGMSWVRQTPDKRLELVATINSNGGTTYYPDSVKGRFTISRDNAKNTLYLQMSSLKSEDSAMYYCARDRDAMDYWGQGTSVTVSS

SEQ ID NO: 86 - protein, 112 aa, Artificial Sequence
  antibody of clostridium botulinum
DVLMTQTPLSLPVSLGDQASISCRSSQSIVNSHGNTYLEWYLQKPGQSPKLLIYKVSNRFSGVPDRFSGSGSGTDFTLKISRVEAEDLGVYYCFQGSHVPWTFGGGTKLEIK

SEQ ID NO: 87 - protein, 113 aa, Artificial Sequence
  antibody of clostridium botulinum
EVQLQQSGPELVKPGASVKISCKASGYTFTDYNMHWVKQSHGKSLEWIGYIYPYNGDTGYNQKFKSKATLTVDNSSSTAYMELRSLTSEDSAVYYCVRSGDYWGQGTTLTVSS

SEQ ID NO: 88 - protein, 112 aa, Artificial Sequence
  antibody of clostridium botulinum
DVLMTQTPLTLSVTIGQPASISCKSSQSLLDSNGKTYLNWLLQRPGQSPSRLIYLVSKLDSGVPDRFTGSGSGTDFTLKISRVEAEDLGVYYCWQGTLFPYTFGGGTKLEIK

SEQ ID NO: 89 - protein, 114 aa, Artificial Sequence
  antibody of clostridium botulinum
QIQLAQSGPELKKPGETVKISCKASGYTFTNYGMSWVKQAPGKGLKWMGWINTYTGEPTYAADFKGRFAFSLETSASTAFLQINNLKNEDTATYFCARGYYDYWGQGTTLTVSS

SEQ ID NO: 90 - protein, 112 aa, Artificial Sequence
  antibody of clostridium botulinum
DVLMTQTPLTLSVTIGQPASISCKSSQSLLDSDGKTYLNWLLQRPGQSPKRLIYLVSKLDSGVPDRFTGSGSGTDFTLKISRVEAEDLGVYYCWQGTHFPRTFGGGTKLEIK